European Patent Application EP 4 397 754 A1, published July 10, 2024. Title: Transesterification enzyme agent comprising lipase as an active ingredient. Applicant: AMANO ENZYME INC. The sequence listing filed with the application follows.

SEQUENCE LISTING (12 sequences)

SEQ ID NO: 1 - DNA, 876 bp, Thermomyces dupontii
  source 1..876: mol_type = other DNA
  CDS 1..876
atgaggagctcgctcgtgctgttcttcgtttctgcgtggacggccttggccagtcctgtccgacgagaggtctcgcaggatctgtttgaccagttcaacctctttgcgcagtactcggcggccgcatactgcgcgaagaacaacgatgccccggcaggtgggaacgtaacgtgcaggggaagtatttgccccgaggtagagaaggcggatgcaacgtttctctactcgtttgaggattctggagttggcgatgtcaccgggttccttgctctcgacaacacgaacagactgatcgtcctctctttccgcggctctcgttccctggaaaactggatcgggaatatcaacttggacttgaaaggaattgacgacatctgctctggctgcaagggacatgacggcttcacttcctcctggaggtccgttgccaataccttgactcagcaagtgcagaatgctgtgagggagcatcccgactaccgcgtcgtcttcactgggcacagcttgggtggtgcattggcaactgtggccggggcatctctgcgtggaaatgggtacgatatagatgtgttctcatatggcgctccccgcgtcggaaacagggcttttgcggaattcctgaccgcacagaccggcggcaccttgtaccgcatcacccacaccaatgatattgtccccagactcccgccacgcgaattgggttacagccattctagcccagagtattggatcacgtctggaaccctcgtcccagtgaccaagaacgatatcgtcaaggtggagggcatcgattccaccgatggaaacaaccagccaaataccccggacattgctgcgcacctatggtacttcgggtcaatggcgacgtgtttgtaa

SEQ ID NO: 2 - protein, 291 aa, Thermomyces dupontii
MRSSLVLFFVSAWTALASPVRREVSQDLFDQFNLFAQYSAAAYCAKNNDAPAGGNVTCRGSICPEVEKADATFLYSFEDSGVGDVTGFLALDNTNRLIVLSFRGSRSLENWIGNINLDLKGIDDICSGCKGHDGFTSSWRSVANTLTQQVQNAVREHPDYRVVFTGHSLGGALATVAGASLRGNGYDIDVFSYGAPRVGNRAFAEFLTAQTGGTLYRITHTNDIVPRLPPRELGYSHSSPEYWITSGTLVPVTKNDIVKVEGIDSTDGNNQPNTPDIAAHLWYFGSMATCL

SEQ ID NO: 3 - DNA, 876 bp, Thermomyces dupontii
  source 1..876: mol_type = other DNA
  CDS 1..876
atgagaggttttctcgtgctgttcttcatctctgcgtggacggccttggccaggcctgttcgacgagaagtctcgcaggatctgctcgatctgttcaacctctttgcacaatactcggcagccgcctactgcgcggaaaacaacgacgctccagtgggctcgaacgtaacgtgctcggagaatgtctgtcccaaggtagaggaggcggacgcaacattcctctattcttttgaagattctggactgggcgatgtcaccggccttctcgcgctcgacaacacgaacaaactgatcgtccttgctttccgcggctctcgctcaatagagaactggatcgggaatctcatcgtcggtctgcgagatatcgacgatatctgctccggctgcgaggggcataccggcttcgtggcttcctggaagtccgtagccaataccctgagaggacaggtcgagaatgccgtgaaggagcatcccgactaccgcgtggtcttcacaggacatagtttgggtggtgcactggcaaccattgctggagccgctctgcgtgggaatgggtataatatcgacgtgttctcatatggcgccccccgcgtcggcaacagggcttttgcagaatttctgaccgcacagaccggtggcaccctgtaccgcatcacccacaccaatgatattgtccccagactcccaccgcgagactggggttacagtcactccagcccagagtactggatcacgtccggcaatgacgccccagtgaccgcaaacgatatcgtcaaggtggagggcattgattccaccgacggtaacaaccagccgaatatcccggacattccttcacatctatggtactttggagccattgcagagtgtgattaa

SEQ ID NO: 4 - protein, 291 aa, Thermomyces dupontii
MRGFLVLFFISAWTALARPVRREVSQDLLDLFNLFAQYSAAAYCAENNDAPVGSNVTCSENVCPKVEEADATFLYSFEDSGLGDVTGLLALDNTNKLIVLAFRGSRSIENWIGNLIVGLRDIDDICSGCEGHTGFVASWKSVANTLRGQVENAVKEHPDYRVVFTGHSLGGALATIAGAALRGNGYNIDVFSYGAPRVGNRAFAEFLTAQTGGTLYRITHTNDIVPRLPPRDWGYSHSSPEYWITSGNDAPVTANDIVKVEGIDSTDGNNQPNIPDIPSHLWYFGAIAECD

SEQ ID NO: 5 - DNA, 1083 bp, Thermomyces dupontii
  source 1..1083: mol_type = genomic DNA
atgaggagctcgctcgtgctgttcttcgtttctgcgtggacggccttggccagtcctgtccgacgaggtatgtaaatcacggggtatacttttcatgcattgcatgtcgaacctgctgtactaagattgcgcgcacagaggtctcgcaggatctgtttgaccagttcaacctctttgcgcagtactcggcggccgcatactgcgcgaagaacaacgatgccccggcaggtgggaacgtaacgtgcaggggaagtatttgccccgaggtagagaaggcggatgcaacgtttctctactcgtttgaggagtaggtgtcaacaagagtacaggcacccgtagtagaaatagcagactaactgggaaatgtagttctggagttggcgatgtcaccgggttccttgctctcgacaacacgaacagactgatcgtcctctctttccgcggctctcgttccctggaaaactggatcgggaatatcaacttggacttgaaaggaattgacgacatctgctctggctgcaagggacatgacggcttcacttcctcctggaggtccgttgccaataccttgactcagcaagtgcagaatgctgtgagggagcatcccgactaccgcgtcgtcttcactgggcacagcttgggtggtgcattggcaactgtggccggggcatctctgcgtggaaatgggtacgatatagatgtggtatgtaggaaaaatgatccccgtggagcggtcatgtggaaatgtgcaggggtgtctaatacacagaccaacagttctcatatggcgctccccgcgtcggaaacagggcttttgcggaattcctgaccgcacagaccggcggcaccttgtaccgcatcacccacaccaatgatattgtccccagactcccgccacgcgaattgggttacagccattctagcccagagtattggatcacgtctggaaccctcgtcccagtgaccaagaacgatatcgtcaaggtggagggcatcgattccaccgatggaaacaaccagccaaataccccggacattgctgcgcacctatggtacttcgggtcaatggcgacgtgtttgtaa

SEQ ID NO: 6 - DNA, 1076 bp, Thermomyces dupontii
  source 1..1076: mol_type = genomic DNA
atgagaggttttctcgtgctgttcttcatctctgcgtggacggccttggccaggcctgttcgacgaggtatggaatcaagggacactttcatgcattgcatgttgaacctgctgttctaagattgttcgcgcagaagtctcgcaggatctgctcgatctgttcaacctctttgcacaatactcggcagccgcctactgcgcggaaaacaacgacgctccagtgggctcgaacgtaacgtgctcggagaatgtctgtcccaaggtagaggaggcggacgcaacattcctctattcttttgaagagtgggtgtcgacgaatatacaaagacagtacctagtctaactgggaaatatgtatatatagttctggactgggcgatgtcaccggccttctcgcgctcgacaacacgaacaaactgatcgtccttgctttccgcggctctcgctcaatagagaactggatcgggaatctcatcgtcggtctgcgagatatcgacgatatctgctccggctgcgaggggcataccggcttcgtggcttcctggaagtccgtagccaataccctgagaggacaggtcgagaatgccgtgaaggagcatcccgactaccgcgtggtcttcacaggacatagtttgggtggtgcactggcaaccattgctggagccgctctgcgtgggaatgggtataatatcgacgtggtatgtggaaatagttccccagacaacgatcatgtggaaacgtgcaggggtgtctaatacacggaccaacagttctcatatggcgccccccgcgtcggcaacagggcttttgcagaatttctgaccgcacagaccggtggcaccctgtaccgcatcacccacaccaatgatattgtccccagactcccaccgcgagactggggttacagtcactccagcccagagtactggatcacgtccggcaatgacgccccagtgaccgcaaacgatatcgtcaaggtggagggcattgattccaccgacggtaacaaccagccgaatatcccggacattccttcacatctatggtactttggagccattgcagagtgtgattaa

SEQ ID NO: 7 - DNA, 35 bp, synthetic construct
  misc_feature 1..35: note = Description of Artificial Sequence: Synthetic DNA
  source 1..35: mol_type = other DNA
atgaggagctcccttgtgctgttcttcatctctgc

SEQ ID NO: 8 - DNA, 34 bp, synthetic construct
  misc_feature 1..34: note = Description of Artificial Sequence: Synthetic DNA
  source 1..34: mol_type = other DNA
ttaatcacactctgcaatggctccaaagtaccat

SEQ ID NO: 9 - DNA, 31 bp, synthetic construct
  misc_feature 1..31: note = Description of Artificial Sequence: Synthetic DNA
  source 1..31: mol_type = other DNA
aggggtgtctaatacacagaccaacagttct

SEQ ID NO: 10 - DNA, 33 bp, synthetic construct
  misc_feature 1..33: note = Description of Artificial Sequence: Synthetic DNA
  source 1..33: mol_type = other DNA
gcacatttccacatgaccgctccacggggatca

SEQ ID NO: 11 - DNA, 31 bp, synthetic construct
  misc_feature 1..31: note = Description of Artificial Sequence: Synthetic DNA
  source 1..31: mol_type = other DNA
ggaatctcatcgtcggtctgcgagatatcga

SEQ ID NO: 12 - DNA, 33 bp, synthetic construct
  misc_feature 1..33: note = Description of Artificial Sequence: Synthetic DNA
  source 1..33: mol_type = other DNA
cgatccagttctctattgagcgagagccgcgga